European Patent Application EP 4 140 495 A1, published March 1, 2023. Title: PHARMACEUTICAL COMPOSITION FOR TREATING CANCER COMPRISING FUSION PROTEIN COMPRISING IL-2 PROTEIN AND CD80 PROTEIN AND ANTICANCER DRUG. Applicant: GI Innovation, Inc. The sequence listing filed with the application follows.

SEQUENCE LISTING (39 sequences)

SEQ ID NO: 1 - protein, 25 aa, Artificial Sequence
  signal peptide (TPA)
MDAMLRGLCCVLLLCGAVFVSPSHA

SEQ ID NO: 2 - protein, 208 aa, Artificial Sequence [sequence omitted]

SEQ ID NO: 3 - protein, 30 aa, Artificial Sequence
  hinge
GSGGGGSGGGGSGGGGSAESKYGPPCPPCP

SEQ ID NO: 4 - protein, 216 aa, Artificial Sequence
  immunoglobulin fc
APEAAGGPSVFLFPPKPKDQLMISRTPEVTCVVVDVSQEDPEVQFNWYVDGVEVHNAKTKPREEQFNSTYRVVSVLTVLHQDWLNGKEYKCKVSNKGLPSSIEKTISKAKGQPREPQVYTLPPSQEEMTKNQVSLTCLVKGFYPSDIAVEWESNGQPENNYKTTPPVLDSDGSFFLYSRLTVDKSRWQEGNVFSCSVLHEALHNHYTQKSLSLSLG

SEQ ID NO: 5 - protein, 5 aa, Artificial Sequence
  linker
GGGGS

SEQ ID NO: 6 - protein, 133 aa, Artificial Sequence
  hIL-2M
APTSSSTKKTQLQLEHLLLDLQMILNGINNYKNPKLTAMLTAKFYMPKKATELKHLQCLEEELKPLEEVLNLAQSKNFHLRPRDLISNINVIVLELKGSETTFMCEYADETATIVEFLNRWITFCQSIISTLT

SEQ ID NO: 7 - protein, 617 aa, Artificial Sequence
  fusion protein comprising variants of IL-2 and fragments of CD80
MDAMLRGLCCVLLLCGAVFVSPSHAVIHVTKEVKEVATLSCGHNVSVEELAQTRIYWQKEKKMVLTMMSGDMNIWPEYKNRTIFDITNNLSIVILALRPSDEGTYECVVLKYEKDAFKREHLAEVTLSVKADFPTPSISDFEIPTSNIRRIICSTSGGFPEPHLSWLENGEELNAINTTVSQDPETELYAVSSKLDFNMTTNHSFMCLIKYGHLRVNQTFNWNTTKQEHFPDNGSGGGGSGGGGSGGGGSAESKYGPPCPPCPAPEAAGGPSVFLFPPKPKDQLMISRTPEVTCVVVDVSQEDPEVQFNWYVDGVEVHNAKTKPREEQFNSTYRVVSVLTVLHQDWLNGKEYKCKVSNKGLPSSIEKTISKAKGQPREPQVYTLPPSQEEMTKNQVSLTCLVKGFYPSDIAVEWESNGQPENNYKTTPPVLDSDGSFFLYSRLTVDKSRWQEGNVFSCSVLHEALHNHYTQKSLSLSLGGGGGSAPTSSSTKKTQLQLEHLLLDLQMILNGINNYKNPKLTAMLTAKFYMPKKATELKHLQCLEEELKPLEEVLNLAQSKNFHLRPRDLISNINVIVLELKGSETTFMCEYADETATIVEFLNRWITFCQSIISTLT

SEQ ID NO: 8 - DNA, 1857 bp, Artificial Sequence
  nucleotiedes coding fusion protein (GI101)
atggatgctatgctgagaggcctgtgttgcgtgctgctgctgtgtggcgctgtgttcgtgtctccttctcacgctgtgatccacgtgaccaaagaagtgaaagaggtcgccacactgtcctgcggccacaacgtttcagtggaagaactggcccagaccaggatctactggcagaaagaaaagaaaatggtgctgaccatgatgtccggcgacatgaacatctggcctgagtacaagaaccggaccatcttcgacatcaccaacaacctgtccatcgtgattctggccctgaggccttctgatgagggcacctatgagtgcgtggtgctgaagtacgagaaggacgccttcaagcgcgagcacctggctgaagtgacactgtccgtgaaggccgactttcccacaccttccatctccgacttcgagatccctacctccaacatccggcggatcatctgttctacctctggcggctttcctgagcctcacctgtcttggctggaaaacggcgaggaactgaacgccatcaacaccaccgtgtctcaggaccccgaaaccgagctgtacgctgtgtcctccaagctggacttcaacatgaccaccaaccacagcttcatgtgcctgattaagtacggccacctgagagtgaaccagaccttcaactggaacaccaccaagcaagagcacttccctgacaatggatctggcggcggaggttctggcggaggtggaagcggaggcggaggatctgctgagtctaagtatggccctccttgtcctccatgtcctgctccagaagctgctggcggaccctctgtgttcctgtttcctccaaagcctaaggaccagctcatgatctctcggacacccgaagtgacctgcgtggtggtggatgtgtctcaagaggaccctgaggtgcagttcaattggtacgtggacggcgtggaagtgcacaacgccaagaccaagcctagagaggaacagttcaactccacctacagagtggtgtccgtgctgaccgtgctgcaccaggattggctgaacggcaaagagtacaagtgcaaggtgtccaacaagggcctgccttccagcatcgaaaagaccatctccaaggctaagggccagcctagggaaccccaggtttacaccctgcctccaagccaagaggaaatgaccaagaaccaggtgtccctgacctgcctggtcaagggcttctacccttccgacattgccgtggaatgggagtccaatggccagcctgagaacaactacaagaccacacctcctgtgctggactccgacggctccttctttctgtactctcgcctgaccgtggacaagtctagatggcaagagggcaacgtgttctcctgctctgtgctgcacgaggccctgcacaatcactacacccagaagtccctgtctctgtctcttggaggtggtggcggttctgcccctaccagctcctctaccaagaaaacccagctccagttggagcatctgctgctggacctccagatgattctgaacgggatcaacaactataagaaccccaagctgaccgccatgctgaccgctaagttctacatgcccaagaaggccaccgagctgaagcacctccagtgcctggaagaagaactgaagcccctggaagaggtgctgaatctggcccagtccaagaacttccacctgaggccacgggacctgatcagcaacatcaacgtgatcgtgctggaactgaagggctccgagacaacctttatgtgcgagtacgccgacgagacagccaccatcgtggaatttctgaaccggtggatcaccttctgccagagcatcatctccacactgacctgatga

SEQ ID NO: 9 - protein, 592 aa, Artificial Sequence
  fusion protein (GI101)
VIHVTKEVKEVATLSCGHNVSVEELAQTRIYWQKEKKMVLTMMSGDMNIWPEYKNRTIFDITNNLSIVILALRPSDEGTYECVVLKYEKDAFKREHLAEVTLSVKADFPTPSISDFEIPTSNIRRIICSTSGGFPEPHLSWLENGEELNAINTTVSQDPETELYAVSSKLDFNMTTNHSFMCLIKYGHLRVNQTFNWNTTKQEHFPDNGSGGGGSGGGGSGGGGSAESKYGPPCPPCPAPEAAGGPSVFLFPPKPKDQLMISRTPEVTCVVVDVSQEDPEVQFNWYVDGVEVHNAKTKPREEQFNSTYRVVSVLTVLHQDWLNGKEYKCKVSNKGLPSSIEKTISKAKGQPREPQVYTLPPSQEEMTKNQVSLTCLVKGFYPSDIAVEWESNGQPENNYKTTPPVLDSDGSFFLYSRLTVDKSRWQEGNVFSCSVLHEALHNHYTQKSLSLSLGGGGGSAPTSSSTKKTQLQLEHLLLDLQMILNGINNYKNPKLTAMLTAKFYMPKKATELKHLQCLEEELKPLEEVLNLAQSKNFHLRPRDLISNINVIVLELKGSETTFMCEYADETATIVEFLNRWITFCQSIISTLT

SEQ ID NO: 10 - protein, 133 aa, Artificial Sequence [sequence omitted]

SEQ ID NO: 11 - protein, 288 aa, Artificial Sequence
  CD80
MGHTRRQGTSPSKCPYLNFFQLLVLAGLSHFCSGVIHVTKEVKEVATLSCGHNVSVEELAQTRIYWQKEKKMVLTMMSGDMNIWPEYKNRTIFDITNNLSIVILALRPSDEGTYECVVLKYEKDAFKREHLAEVTLSVKADFPTPSISDFEIPTSNIRRIICSTSGGFPEPHLSWLENGEELNAINTTVSQDPETELYAVSSKLDFNMTTNHSFMCLIKYGHLRVNQTFNWNTTKQEHFPDNLLPSWAITLISVNGIFVICCLTYCFAPRCRERRRNERLRRESVRPV

SEQ ID NO: 12 - protein, 215 aa, Artificial Sequence
  modified Fc
SHTQPLGVFLFPPKPKDTLMISRTPEVTCVVVDVSQEDPEVQFNWYVDGVEVHNAKTKPREEQFNSTYRVVSVLTVLHQDWLNGKEYKCKVSNKGLPSSIEKTISKAKGQPREPQVYTLPPSQEEMTKNQVSLTCLVKGFYPSDIAVEWESNGQPENNYKTTPPVLDSDGSFFLYSRLTVDKSRWQEGNVFSCSVMHEALHNHYTQKSLSLSLGK

SEQ ID NO: 13 - protein, 306 aa, Artificial Sequence
  mCD80
MACNCQLMQDTPLLKFPCPRLILLFVLLIRLSQVSSDVDEQLSKSVKDKVLLPCRYNSPHEDESEDRIYWQKHDKVVLSVIAGKLKVWPEYKNRTLYDNTTYSLIILGLVLSDRGTYSCVVQKKERGTYEVKHLALVKLSIKADFSTPNITESGNPSADTKRITCFASGGFPKPRFSWLENGRELPGINTTISQDPESELYTISSQLDFNTTRNHTIKCLIKYGDAHVSEDFTWEKPPEDPPDSKNTLVLFGAGFGAVITVVVIVVIIKCFCKHRSCFRRNEASRETNNSLTFGPEEALAEQTVFL

SEQ ID NO: 14 - DNA, 1848 bp, Artificial Sequence
  nucleotiedes coding fusion protein (mGI101)
atggatgctatgctgagaggcctgtgttgcgtgctgctgctgtgtggcgctgtgttcgtgtctccttctcacgctgtggacgagcagctctccaagtccgtgaaggataaggtcctgctgccttgccggtacaactctcctcacgaggacgagtctgaggaccggatctactggcagaaacacgacaaggtggtgctgtccgtgatcgccggaaagctgaaagtgtggcctgagtacaagaacaggaccctgtacgacaacaccacctacagcctgatcatcctgggcctcgtgctgagcgatagaggcacctattcttgcgtggtgcagaagaaagagcggggcacctacgaagtgaagcacctggctctggtcaagctgtccatcaaggccgacttcagcacccctaacatcaccgagtctggcaacccttccgccgacaccaagagaatcacctgtttcgcctctggcggcttccctaagcctcggttctcttggctggaaaacggcagagagctgcccggcatcaataccaccatttctcaggacccagagtccgagctgtacaccatctccagccagctcgactttaacaccaccagaaaccacaccatcaagtgcctgattaagtacggcgacgcccacgtgtccgaggactttacttgggagaaacctcctgaggaccctcctgactctggatctggcggcggaggttctggcggaggtggaagcggaggcggaggatctgctgagtctaagtatggccctccttgtcctccatgtcctgctccagaagctgctggcggaccctctgtgttcctgtttcctccaaagcctaaggaccagctcatgatctctcggacccctgaagtgacctgcgtggtggtggatgtgtctcaagaggaccctgaggtgcagttcaattggtacgtggacggcgtggaagtgcacaacgccaagaccaagcctagagaggaacagttcaactccacctatagagtggtgtccgtgctgaccgtgctgcaccaggattggctgaacggcaaagagtacaagtgcaaggtgtccaacaagggcctgccttccagcatcgaaaagaccatcagcaaggctaagggccagcctagggaaccccaggtttacaccctgcctccaagccaagaggaaatgaccaagaaccaggtgtccctgacctgcctggtcaagggcttctacccttccgacattgccgtggaatgggagtccaatggccagcctgagaacaactacaagaccacacctcctgtgctggactccgacggctccttctttctgtactctcgcctgaccgtggacaagtctaggtggcaagagggcaacgtgttctcctgctctgtgctgcacgaggctctgcacaaccactacacccagaagtccctgtctctgtctcttggaggtggtggcggttctgcccctacctccagctctaccaagaaaacccagctccagttggagcatctgctgctggacctccagatgatcctgaatggcatcaacaattacaagaaccccaagctgaccgccatgctgaccgctaagttctacatgcccaagaaggccaccgagctgaagcacttgcagtgcctggaagaggaactgaagcccctggaagaagtgctgaatctggcccagtccaagaacttccacctgaggcctagggacctgatctccaacatcaacgtgatcgtgctggaactgaaaggctccgagacaaccttcatgtgcgagtacgccgacgagacagccaccatcgtggaatttctgaaccggtggatcaccttctgccagagcatcatctccacactgacc

SEQ ID NO: 15 - protein, 616 aa, Artificial Sequence
  fusion protein (mGI101)
MDAMLRGLCCVLLLCGAVFVSPSHAVDEQLSKSVKDKVLLPCRYNSPHEDESEDRIYWQKHDKVVLSVIAGKLKVWPEYKNRTLYDNTTYSLIILGLVLSDRGTYSCVVQKKERGTYEVKHLALVKLSIKADFSTPNITESGNPSADTKRITCFASGGFPKPRFSWLENGRELPGINTTISQDPESELYTISSQLDFNTTRNHTIKCLIKYGDAHVSEDFTWEKPPEDPPDSGSGGGGSGGGGSGGGGSAESKYGPPCPPCPAPEAAGGPSVFLFPPKPKDQLMISRTPEVTCVVVDVSQEDPEVQFNWYVDGVEVHNAKTKPREEQFNSTYRVVSVLTVLHQDWLNGKEYKCKVSNKGLPSSIEKTISKAKGQPREPQVYTLPPSQEEMTKNQVSLTCLVKGFYPSDIAVEWESNGQPENNYKTTPPVLDSDGSFFLYSRLTVDKSRWQEGNVFSCSVLHEALHNHYTQKSLSLSLGGGGGSAPTSSSTKKTQLQLEHLLLDLQMILNGINNYKNPKLTAMLTAKFYMPKKATELKHLQCLEEELKPLEEVLNLAQSKNFHLRPRDLISNINVIVLELKGSETTFMCEYADETATIVEFLNRWITFCQSIISTLT

SEQ ID NO: 16 - DNA, 1437 bp, Artificial Sequence
  nucleotiedes coding fusion protein (GI101C1)
atggatgctatgctgagaggcctgtgttgcgtgctgctgctgtgtggcgctgtgttcgtgtctccttctcacgctgtgatccacgtgaccaaagaagtgaaagaggtcgccacactgtcctgcggccacaacgtttcagtggaagaactggcccagaccaggatctactggcagaaagaaaagaaaatggtgctgaccatgatgtccggcgacatgaacatctggcctgagtacaagaaccggaccatcttcgacatcaccaacaacctgtccatcgtgattctggccctgaggccttctgatgagggcacctatgagtgcgtggtgctgaagtacgagaaggacgccttcaagcgcgagcacctggctgaagtgacactgtccgtgaaggccgactttcccacaccttccatctccgacttcgagatccctacctccaacatccggcggatcatctgttctacctctggcggctttcctgagcctcacctgtcttggctggaaaacggcgaggaactgaacgccatcaacaccaccgtgtctcaggaccccgaaaccgagctgtacgctgtgtcctccaagctggacttcaacatgaccaccaaccacagcttcatgtgcctgattaagtacggccacctgagagtgaaccagaccttcaactggaacaccaccaagcaagagcacttccctgacaatggatctggcggcggaggttctggcggaggtggaagcggaggcggaggatctgctgagtctaagtatggccctccttgtcctccatgtcctgctccagaagctgctggcggaccctctgtgttcctgtttcctccaaagcctaaggaccagctcatgatctctcggacacccgaagtgacctgcgtggtggtggatgtgtctcaagaggaccctgaggtgcagttcaattggtacgtggacggcgtggaagtgcacaacgccaagaccaagcctagagaggaacagttcaactccacctacagagtggtgtccgtgctgaccgtgctgcaccaggattggctgaacggcaaagagtacaagtgcaaggtgtccaacaagggcctgccttccagcatcgaaaagaccatctccaaggctaagggccagcctagggaaccccaggtttacaccctgcctccaagccaagaggaaatgaccaagaaccaggtgtccctgacctgcctggtcaagggcttctacccttccgacattgccgtggaatgggagtccaatggccagcctgagaacaactacaagaccacacctcctgtgctggactccgacggctccttctttctgtactctcgcctgaccgtggacaagtctaggtggcaagagggcaacgtgttctcctgctctgtgctgcacgaggccctgcacaatcactacacccagaagtccctgtctctgtccctgggc

SEQ ID NO: 17 - protein, 454 aa, Artificial Sequence
  fusion protein (GI101C1)
VIHVTKEVKEVATLSCGHNVSVEELAQTRIYWQKEKKMVLTMMSGDMNIWPEYKNRTIFDITNNLSIVILALRPSDEGTYECVVLKYEKDAFKREHLAEVTLSVKADFPTPSISDFEIPTSNIRRIICSTSGGFPEPHLSWLENGEELNAINTTVSQDPETELYAVSSKLDFNMTTNHSFMCLIKYGHLRVNQTFNWNTTKQEHFPDNGSGGGGSGGGGSGGGGSAESKYGPPCPPCPAPEAAGGPSVFLFPPKPKDQLMISRTPEVTCVVVDVSQEDPEVQFNWYVDGVEVHNAKTKPREEQFNSTYRVVSVLTVLHQDWLNGKEYKCKVSNKGLPSSIEKTISKAKGQPREPQVYTLPPSQEEMTKNQVSLTCLVKGFYPSDIAVEWESNGQPENNYKTTPPVLDSDGSFFLYSRLTVDKSRWQEGNVFSCSVLHEALHNHYTQKSLSLSLG

SEQ ID NO: 18 - DNA, 1176 bp, Artificial Sequence
  nucleotiedes coding fusion protein (GI101C2)
atggatgctatgctgagaggcctgtgttgcgtgctgctgctgtgtggcgctgtgttcgtgtctccatctcacgccgctgagtctaagtacggccctccttgtcctccatgtcctgctccagaagctgctggcggaccctctgtgttcctgtttcctccaaagcctaaggaccagctcatgatctctcggacccctgaagtgacctgcgtggtggtggatgtgtctcaagaggaccctgaggtgcagttcaattggtacgtggacggcgtggaagtgcacaacgccaagaccaagcctagagaggaacagttcaactccacctacagagtggtgtccgtgctgaccgtgctgcaccaggattggctgaacggcaaagagtacaagtgcaaggtgtccaacaagggcctgccttccagcatcgaaaagaccatctccaaggctaagggccagcctagggaaccccaggtttacaccctgcctccaagccaagaggaaatgaccaagaaccaggtgtccctgacctgcctggtcaagggcttctacccttccgacattgccgtggaatgggagtccaatggccagcctgagaacaactacaagaccacacctcctgtgctggactccgacggctccttctttctgtactctcgcctgaccgtggacaagtctaggtggcaagagggcaacgtgttctcctgctctgtgctgcacgaggccctgcacaatcactacacccagaagtccctgtctctgtctcttggcggaggcggaggatctgctcctacctccagctccaccaagaaaacccagctccagttggagcatctgctgctggacctccagatgatcctgaatggcatcaacaattacaagaaccccaagctgaccgccatgctgaccgctaagttctacatgcccaagaaggccaccgagctgaagcacctccagtgcctggaagaggaactgaagcccctggaagaagtgctgaatctggcccagtccaagaacttccacctgaggcctagggacctgatctccaacatcaacgtgatcgtgctggaactgaaaggctccgagacaaccttcatgtgcgagtacgccgacgagacagccaccatcgtggaatttctgaaccggtggatcaccttctgccagtccatcatctccacactgacc

SEQ ID NO: 19 - protein, 367 aa, Artificial Sequence
  fusion protein (GI101C2)
AESKYGPPCPPCPAPEAAGGPSVFLFPPKPKDQLMISRTPEVTCVVVDVSQEDPEVQFNWYVDGVEVHNAKTKPREEQFNSTYRVVSVLTVLHQDWLNGKEYKCKVSNKGLPSSIEKTISKAKGQPREPQVYTLPPSQEEMTKNQVSLTCLVKGFYPSDIAVEWESNGQPENNYKTTPPVLDSDGSFFLYSRLTVDKSRWQEGNVFSCSVLHEALHNHYTQKSLSLSLGGGGGSAPTSSSTKKTQLQLEHLLLDLQMILNGINNYKNPKLTAMLTAKFYMPKKATELKHLQCLEEELKPLEEVLNLAQSKNFHLRPRDLISNINVIVLELKGSETTFMCEYADETATIVEFLNRWITFCQSIISTLT

SEQ ID NO: 20 - DNA, 1434 bp, Artificial Sequence
  nucleotiedes coding fusion protein (mGI101C1)
atggatgctatgctgagaggcctgtgttgcgtgctgctgctgtgtggcgctgtgttcgtgtctccttctcacgctgtggacgagcagctctccaagtccgtgaaggataaggtcctgctgccttgccggtacaactctcctcacgaggacgagtctgaggaccggatctactggcagaaacacgacaaggtggtgctgtccgtgatcgccggaaagctgaaagtgtggcctgagtacaagaacaggaccctgtacgacaacaccacctacagcctgatcatcctgggcctcgtgctgagcgatagaggcacctattcttgcgtggtgcagaagaaagagcggggcacctacgaagtgaagcacctggctctggtcaagctgtccatcaaggccgacttcagcacccctaacatcaccgagtctggcaacccttccgccgacaccaagagaatcacctgtttcgcctctggcggcttccctaagcctcggttctcttggctggaaaacggcagagagctgcccggcatcaataccaccatttctcaggacccagagtccgagctgtacaccatctccagccagctcgactttaacaccaccagaaaccacaccatcaagtgcctgattaagtacggcgacgcccacgtgtccgaggactttacttgggagaaacctcctgaggaccctcctgactctggatctggcggcggaggttctggcggaggtggaagcggaggcggaggatctgctgagtctaagtatggccctccttgtcctccatgtcctgctccagaagctgctggcggaccctctgtgttcctgtttcctccaaagcctaaggaccagctcatgatctctcggacccctgaagtgacctgcgtggtggtggatgtgtctcaagaggaccctgaggtgcagttcaattggtacgtggacggcgtggaagtgcacaacgccaagaccaagcctagagaggaacagttcaactccacctatagagtggtgtccgtgctgaccgtgctgcaccaggattggctgaacggcaaagagtacaagtgcaaggtgtccaacaagggcctgccttccagcatcgaaaagaccatcagcaaggctaagggccagcctagggaaccccaggtttacaccctgcctccaagccaagaggaaatgaccaagaaccaggtgtccctgacctgcctggtcaagggcttctacccttccgacattgccgtggaatgggagtccaatggccagcctgagaacaactacaagaccacacctcctgtgctggactccgacggctccttctttctgtactctcgcctgaccgtggacaagtctaggtggcaagagggcaacgtgttctcctgctctgtgctgcacgaggctctgcacaaccactacacccagaagtccctgtctctgtccctgggc

SEQ ID NO: 21 - protein, 478 aa, Artificial Sequence
  fusion protein (mGI101C1)
MDAMLRGLCCVLLLCGAVFVSPSHAVDEQLSKSVKDKVLLPCRYNSPHEDESEDRIYWQKHDKVVLSVIAGKLKVWPEYKNRTLYDNTTYSLIILGLVLSDRGTYSCVVQKKERGTYEVKHLALVKLSIKADFSTPNITESGNPSADTKRITCFASGGFPKPRFSWLENGRELPGINTTISQDPESELYTISSQLDFNTTRNHTIKCLIKYGDAHVSEDFTWEKPPEDPPDSGSGGGGSGGGGSGGGGSAESKYGPPCPPCPAPEAAGGPSVFLFPPKPKDQLMISRTPEVTCVVVDVSQEDPEVQFNWYVDGVEVHNAKTKPREEQFNSTYRVVSVLTVLHQDWLNGKEYKCKVSNKGLPSSIEKTISKAKGQPREPQVYTLPPSQEEMTKNQVSLTCLVKGFYPSDIAVEWESNGQPENNYKTTPPVLDSDGSFFLYSRLTVDKSRWQEGNVFSCSVLHEALHNHYTQKSLSLSLG

SEQ ID NO: 22 - protein, 133 aa, Artificial Sequence
  variants of IL-2 (3M, M45)
APTSSSTKKTQLQLEHLLLDLQMILNGINNYKNPKLTAMLTAKFAMPKKATELKHLQCLEEELKPLEEVLNLAQSKNFHLRPRDLISNINVIVLELKGSETTFMCEYADETATIVEFLNRWITFCQSIISTLT

SEQ ID NO: 23 - protein, 133 aa, Artificial Sequence
  variants of IL-2 (3M, M61)
APTSSSTKKTQLQLEHLLLDLQMILNGINNYKNPKLTAMLTAKFYMPKKATELKHLQCLERELKPLEEVLNLAQSKNFHLRPRDLISNINVIVLELKGSETTFMCEYADETATIVEFLNRWITFCQSIISTLT

SEQ ID NO: 24 - protein, 133 aa, Artificial Sequence
  variants of IL-2 (3M, M72)
APTSSSTKKTQLQLEHLLLDLQMILNGINNYKNPKLTAMLTAKFYMPKKATELKHLQCLEEELKPLEEVLNGAQSKNFHLRPRDLISNINVIVLELKGSETTFMCEYADETATIVEFLNRWITFCQSIISTLT

SEQ ID NO: 25 - DNA, 1851 bp, Artificial Sequence
  nucleotiedes coding fusion protein (GI102-M45)
atggatgctatgctgagaggcctgtgttgcgtgctgctgctgtgtggcgctgtgttcgtgtctccttctcacgctgtgatccacgtgaccaaagaagtgaaagaggtcgccacactgtcctgcggccacaacgtttcagtggaagaactggcccagaccaggatctactggcagaaagaaaagaaaatggtgctgaccatgatgtccggcgacatgaacatctggcctgagtacaagaaccggaccatcttcgacatcaccaacaacctgtccatcgtgattctggccctgaggccttctgatgagggcacctatgagtgcgtggtgctgaagtacgagaaggacgccttcaagcgcgagcacctggctgaagtgacactgtccgtgaaggccgactttcccacaccttccatctccgacttcgagatccctacctccaacatccggcggatcatctgttctacctctggcggctttcctgagcctcacctgtcttggctggaaaacggcgaggaactgaacgccatcaacaccaccgtgtctcaggaccccgaaaccgagctgtacgctgtgtcctccaagctggacttcaacatgaccaccaaccacagcttcatgtgcctgattaagtacggccacctgagagtgaaccagaccttcaactggaacaccaccaagcaagagcacttccctgacaatggatctggcggcggaggttctggcggaggtggaagcggaggcggaggatctgctgagtctaagtatggccctccttgtcctccatgtcctgctccagaagctgctggcggaccctctgtgttcctgtttcctccaaagcctaaggaccagctcatgatctctcggacacccgaagtgacctgcgtggtggtggatgtgtctcaagaggaccctgaggtgcagttcaattggtacgtggacggcgtggaagtgcacaacgccaagaccaagcctagagaggaacagttcaactccacctacagagtggtgtccgtgctgaccgtgctgcaccaggattggctgaacggcaaagagtacaagtgcaaggtgtccaacaagggcctgccttccagcatcgaaaagaccatctccaaggctaagggccagcctagggaaccccaggtttacaccctgcctccaagccaagaggaaatgaccaagaaccaggtgtccctgacctgcctggtcaagggcttctacccttccgacattgccgtggaatgggagtccaatggccagcctgagaacaactacaagaccacacctcctgtgctggactccgacggctccttctttctgtactctcgcctgaccgtggacaagtctagatggcaagagggcaacgtgttctcctgctctgtgctgcacgaggccctgcacaatcactacacccagaagtccctgtctctgtctcttggaggtggtggcggttctgcccctaccagctcctctaccaagaaaacccagctccagttggagcatctgctgctggacctccagatgattctgaacgggatcaacaactataagaaccccaagctgaccgccatgctgaccgctaagttcgccatgcccaagaaggccaccgagctgaagcacctccagtgcctggaagaagaactgaagcccctggaagaggtgctgaatctggcccagtccaagaacttccacctgaggccacgggacctgatcagcaacatcaacgtgatcgtgctggaactgaagggctccgagacaacctttatgtgcgagtacgccgacgagacagccaccatcgtggaatttctgaaccggtggatcaccttctgccagagcatcatctccacactgacc

SEQ ID NO: 26 - protein, 592 aa, Artificial Sequence
  fusion protein (GI102-M45)
VIHVTKEVKEVATLSCGHNVSVEELAQTRIYWQKEKKMVLTMMSGDMNIWPEYKNRTIFDITNNLSIVILALRPSDEGTYECVVLKYEKDAFKREHLAEVTLSVKADFPTPSISDFEIPTSNIRRIICSTSGGFPEPHLSWLENGEELNAINTTVSQDPETELYAVSSKLDFNMTTNHSFMCLIKYGHLRVNQTFNWNTTKQEHFPDNGSGGGGSGGGGSGGGGSAESKYGPPCPPCPAPEAAGGPSVFLFPPKPKDQLMISRTPEVTCVVVDVSQEDPEVQFNWYVDGVEVHNAKTKPREEQFNSTYRVVSVLTVLHQDWLNGKEYKCKVSNKGLPSSIEKTISKAKGQPREPQVYTLPPSQEEMTKNQVSLTCLVKGFYPSDIAVEWESNGQPENNYKTTPPVLDSDGSFFLYSRLTVDKSRWQEGNVFSCSVLHEALHNHYTQKSLSLSLGGGGGSAPTSSSTKKTQLQLEHLLLDLQMILNGINNYKNPKLTAMLTAKFAMPKKATELKHLQCLEEELKPLEEVLNLAQSKNFHLRPRDLISNINVIVLELKGSETTFMCEYADETATIVEFLNRWITFCQSIISTLT

SEQ ID NO: 27 - DNA, 1851 bp, Artificial Sequence
  nucleotiedes coding fusion protein (GI102-M61)
atggatgctatgctgagaggcctgtgttgcgtgctgctgctgtgtggcgctgtgttcgtgtctccttctcacgctgtgatccacgtgaccaaagaagtgaaagaggtcgccacactgtcctgcggccacaacgtttcagtggaagaactggcccagaccaggatctactggcagaaagaaaagaaaatggtgctgaccatgatgtccggcgacatgaacatctggcctgagtacaagaaccggaccatcttcgacatcaccaacaacctgtccatcgtgattctggccctgaggccttctgatgagggcacctatgagtgcgtggtgctgaagtacgagaaggacgccttcaagcgcgagcacctggctgaagtgacactgtccgtgaaggccgactttcccacaccttccatctccgacttcgagatccctacctccaacatccggcggatcatctgttctacctctggcggctttcctgagcctcacctgtcttggctggaaaacggcgaggaactgaacgccatcaacaccaccgtgtctcaggaccccgaaaccgagctgtacgctgtgtcctccaagctggacttcaacatgaccaccaaccacagcttcatgtgcctgattaagtacggccacctgagagtgaaccagaccttcaactggaacaccaccaagcaagagcacttccctgacaatggatctggcggcggaggttctggcggaggtggaagcggaggcggaggatctgctgagtctaagtatggccctccttgtcctccatgtcctgctccagaagctgctggcggaccctctgtgttcctgtttcctccaaagcctaaggaccagctcatgatctctcggacacccgaagtgacctgcgtggtggtggatgtgtctcaagaggaccctgaggtgcagttcaattggtacgtggacggcgtggaagtgcacaacgccaagaccaagcctagagaggaacagttcaactccacctacagagtggtgtccgtgctgaccgtgctgcaccaggattggctgaacggcaaagagtacaagtgcaaggtgtccaacaagggcctgccttccagcatcgaaaagaccatctccaaggctaagggccagcctagggaaccccaggtttacaccctgcctccaagccaagaggaaatgaccaagaaccaggtgtccctgacctgcctggtcaagggcttctacccttccgacattgccgtggaatgggagtccaatggccagcctgagaacaactacaagaccacacctcctgtgctggactccgacggctccttctttctgtactctcgcctgaccgtggacaagtctagatggcaagagggcaacgtgttctcctgctctgtgctgcacgaggccctgcacaatcactacacccagaagtccctgtctctgtctcttggaggtggtggcggttctgcccctaccagctcctctaccaagaaaacccagctccagttggagcatctgctgctggacctccagatgattctgaacgggatcaacaactataagaaccccaagctgaccgccatgctgaccgctaagttctacatgcccaagaaggccaccgagctgaagcacctccagtgcctggaaagggaactgaagcccctggaagaggtgctgaatctggcccagtccaagaacttccacctgaggccacgggacctgatcagcaacatcaacgtgatcgtgctggaactgaagggctccgagacaacctttatgtgcgagtacgccgacgagacagccaccatcgtggaatttctgaaccggtggatcaccttctgccagagcatcatctccacactgacc

SEQ ID NO: 28 - protein, 592 aa, Artificial Sequence
  fusion protein (GI102-M61)
VIHVTKEVKEVATLSCGHNVSVEELAQTRIYWQKEKKMVLTMMSGDMNIWPEYKNRTIFDITNNLSIVILALRPSDEGTYECVVLKYEKDAFKREHLAEVTLSVKADFPTPSISDFEIPTSNIRRIICSTSGGFPEPHLSWLENGEELNAINTTVSQDPETELYAVSSKLDFNMTTNHSFMCLIKYGHLRVNQTFNWNTTKQEHFPDNGSGGGGSGGGGSGGGGSAESKYGPPCPPCPAPEAAGGPSVFLFPPKPKDQLMISRTPEVTCVVVDVSQEDPEVQFNWYVDGVEVHNAKTKPREEQFNSTYRVVSVLTVLHQDWLNGKEYKCKVSNKGLPSSIEKTISKAKGQPREPQVYTLPPSQEEMTKNQVSLTCLVKGFYPSDIAVEWESNGQPENNYKTTPPVLDSDGSFFLYSRLTVDKSRWQEGNVFSCSVLHEALHNHYTQKSLSLSLGGGGGSAPTSSSTKKTQLQLEHLLLDLQMILNGINNYKNPKLTAMLTAKFYMPKKATELKHLQCLERELKPLEEVLNLAQSKNFHLRPRDLISNINVIVLELKGSETTFMCEYADETATIVEFLNRWITFCQSIISTLT

SEQ ID NO: 29 - DNA, 1857 bp, Artificial Sequence
  nucleotiedes coding fusion protein (GI102-M72)
atggatgctatgctgagaggcctgtgttgcgtgctgctgctgtgtggcgctgtgttcgtgtctccttctcacgctgtgatccacgtgaccaaagaagtgaaagaggtcgccacactgtcctgcggccacaacgtttcagtggaagaactggcccagaccaggatctactggcagaaagaaaagaaaatggtgctgaccatgatgtccggcgacatgaacatctggcctgagtacaagaaccggaccatcttcgacatcaccaacaacctgtccatcgtgattctggccctgaggccttctgatgagggcacctatgagtgcgtggtgctgaagtacgagaaggacgccttcaagcgcgagcacctggctgaagtgacactgtccgtgaaggccgactttcccacaccttccatctccgacttcgagatccctacctccaacatccggcggatcatctgttctacctctggcggctttcctgagcctcacctgtcttggctggaaaacggcgaggaactgaacgccatcaacaccaccgtgtctcaggaccccgaaaccgagctgtacgctgtgtcctccaagctggacttcaacatgaccaccaaccacagcttcatgtgcctgattaagtacggccacctgagagtgaaccagaccttcaactggaacaccaccaagcaagagcacttccctgacaatggatctggcggcggaggttctggcggaggtggaagcggaggcggaggatctgctgagtctaagtatggccctccttgtcctccatgtcctgctccagaagctgctggcggaccctctgtgttcctgtttcctccaaagcctaaggaccagctcatgatctctcggacacccgaagtgacctgcgtggtggtggatgtgtctcaagaggaccctgaggtgcagttcaattggtacgtggacggcgtggaagtgcacaacgccaagaccaagcctagagaggaacagttcaactccacctacagagtggtgtccgtgctgaccgtgctgcaccaggattggctgaacggcaaagagtacaagtgcaaggtgtccaacaagggcctgccttccagcatcgaaaagaccatctccaaggctaagggccagcctagggaaccccaggtttacaccctgcctccaagccaagaggaaatgaccaagaaccaggtgtccctgacctgcctggtcaagggcttctacccttccgacattgccgtggaatgggagtccaatggccagcctgagaacaactacaagaccacacctcctgtgctggactccgacggctccttctttctgtactctcgcctgaccgtggacaagtctagatggcaagagggcaacgtgttctcctgctctgtgctgcacgaggccctgcacaatcactacacccagaagtccctgtctctgtctcttggaggtggtggcggttctgcccctaccagctcctctaccaagaaaacccagctccagttggagcatctgctgctggacctccagatgattctgaacgggatcaacaactataagaaccccaagctgaccgccatgctgaccgctaagttctacatgcccaagaaggccaccgagctgaagcacctccagtgcctggaagaagaactgaagcccctggaagaggtgctgaatggggcccagtccaagaacttccacctgaggccacgggacctgatcagcaacatcaacgtgatcgtgctggaactgaagggctccgagacaacctttatgtgcgagtacgccgacgagacagccaccatcgtggaatttctgaaccggtggatcaccttctgccagagcatcatctccacactgacctgatga

SEQ ID NO: 30 - protein, 592 aa, Artificial Sequence
  fusion protein (GI102-M72)
VIHVTKEVKEVATLSCGHNVSVEELAQTRIYWQKEKKMVLTMMSGDMNIWPEYKNRTIFDITNNLSIVILALRPSDEGTYECVVLKYEKDAFKREHLAEVTLSVKADFPTPSISDFEIPTSNIRRIICSTSGGFPEPHLSWLENGEELNAINTTVSQDPETELYAVSSKLDFNMTTNHSFMCLIKYGHLRVNQTFNWNTTKQEHFPDNGSGGGGSGGGGSGGGGSAESKYGPPCPPCPAPEAAGGPSVFLFPPKPKDQLMISRTPEVTCVVVDVSQEDPEVQFNWYVDGVEVHNAKTKPREEQFNSTYRVVSVLTVLHQDWLNGKEYKCKVSNKGLPSSIEKTISKAKGQPREPQVYTLPPSQEEMTKNQVSLTCLVKGFYPSDIAVEWESNGQPENNYKTTPPVLDSDGSFFLYSRLTVDKSRWQEGNVFSCSVLHEALHNHYTQKSLSLSLGGGGGSAPTSSSTKKTQLQLEHLLLDLQMILNGINNYKNPKLTAMLTAKFYMPKKATELKHLQCLEEELKPLEEVLNGAQSKNFHLRPRDLISNINVIVLELKGSETTFMCEYADETATIVEFLNRWITFCQSIISTLT

SEQ ID NO: 31 - DNA, 1851 bp, Artificial Sequence
  nucleotiedes coding fusion protein (GI101w)
atggatgctatgctgagaggcctgtgttgcgtgctgctgctgtgtggcgctgtgttcgtgtctccttctcacgctgtgatccacgtgaccaaagaagtgaaagaggtcgccacactgtcctgcggccacaacgtttcagtggaagaactggcccagaccaggatctactggcagaaagaaaagaaaatggtgctgaccatgatgtccggcgacatgaacatctggcctgagtacaagaaccggaccatcttcgacatcaccaacaacctgtccatcgtgattctggccctgaggccttctgatgagggcacctatgagtgcgtggtgctgaagtacgagaaggacgccttcaagcgcgagcacctggctgaagtgacactgtccgtgaaggccgactttcccacaccttccatctccgacttcgagatccctacctccaacatccggcggatcatctgttctacctctggcggctttcctgagcctcacctgtcttggctggaaaacggcgaggaactgaacgccatcaacaccaccgtgtctcaggaccccgaaaccgagctgtacgctgtgtcctccaagctggacttcaacatgaccaccaaccacagcttcatgtgcctgattaagtacggccacctgagagtgaaccagaccttcaactggaacaccaccaagcaagagcacttccctgacaatggatctggcggcggaggttctggcggaggtggaagcggaggcggaggatctgctgagtctaagtatggccctccttgtcctccatgtcctgctccagaagctgctggcggaccctctgtgttcctgtttcctccaaagcctaaggaccagctcatgatctctcggacacccgaagtgacctgcgtggtggtggatgtgtctcaagaggaccctgaggtgcagttcaattggtacgtggacggcgtggaagtgcacaacgccaagaccaagcctagagaggaacagttcaactccacctacagagtggtgtccgtgctgaccgtgctgcaccaggattggctgaacggcaaagagtacaagtgcaaggtgtccaacaagggcctgccttccagcatcgaaaagaccatctccaaggctaagggccagcctagggaaccccaggtttacaccctgcctccaagccaagaggaaatgaccaagaaccaggtgtccctgacctgcctggtcaagggcttctacccttccgacattgccgtggaatgggagtccaatggccagcctgagaacaactacaagaccacacctcctgtgctggactccgacggctccttctttctgtactctcgcctgaccgtggacaagtctagatggcaagagggcaacgtgttctcctgctctgtgctgcacgaggccctgcacaatcactacacccagaagtccctgtctctgtctcttggaggtggtggcggttctgcccctaccagctcctctaccaagaaaacccagctccagttggagcatctgctgctggacctccagatgattctgaacgggatcaacaactataagaaccccaagctgacccgcatgctgacctttaagttctacatgcccaagaaggccaccgagctgaagcacctccagtgcctggaagaagaactgaagcccctggaagaggtgctgaatctggcccagtccaagaacttccacctgaggccacgggacctgatcagcaacatcaacgtgatcgtgctggaactgaagggctccgagacaacctttatgtgcgagtacgccgacgagacagccaccatcgtggaatttctgaaccggtggatcaccttctgccagagcatcatctccacactgacc

SEQ ID NO: 32 - protein, 592 aa, Artificial Sequence
  fusion protein (GI101w)
VIHVTKEVKEVATLSCGHNVSVEELAQTRIYWQKEKKMVLTMMSGDMNIWPEYKNRTIFDITNNLSIVILALRPSDEGTYECVVLKYEKDAFKREHLAEVTLSVKADFPTPSISDFEIPTSNIRRIICSTSGGFPEPHLSWLENGEELNAINTTVSQDPETELYAVSSKLDFNMTTNHSFMCLIKYGHLRVNQTFNWNTTKQEHFPDNGSGGGGSGGGGSGGGGSAESKYGPPCPPCPAPEAAGGPSVFLFPPKPKDQLMISRTPEVTCVVVDVSQEDPEVQFNWYVDGVEVHNAKTKPREEQFNSTYRVVSVLTVLHQDWLNGKEYKCKVSNKGLPSSIEKTISKAKGQPREPQVYTLPPSQEEMTKNQVSLTCLVKGFYPSDIAVEWESNGQPENNYKTTPPVLDSDGSFFLYSRLTVDKSRWQEGNVFSCSVLHEALHNHYTQKSLSLSLGGGGGSAPTSSSTKKTQLQLEHLLLDLQMILNGINNYKNPKLTRMLTFKFYMPKKATELKHLQCLEEELKPLEEVLNLAQSKNFHLRPRDLISNINVIVLELKGSETTFMCEYADETATIVEFLNRWITFCQSIISTLT

SEQ ID NO: 33 - DNA, 1848 bp, Artificial Sequence
  nucleotiedes coding fusion protein (mGI102-M61)
atggatgctatgctgagaggcctgtgttgcgtgctgctgctgtgtggcgctgtgttcgtgtctccttctcacgctgtggacgagcagctctccaagtccgtgaaggataaggtcctgctgccttgccggtacaactctcctcacgaggacgagtctgaggaccggatctactggcagaaacacgacaaggtggtgctgtccgtgatcgccggaaagctgaaagtgtggcctgagtacaagaacaggaccctgtacgacaacaccacctacagcctgatcatcctgggcctcgtgctgagcgatagaggcacctattcttgcgtggtgcagaagaaagagcggggcacctacgaagtgaagcacctggctctggtcaagctgtccatcaaggccgacttcagcacccctaacatcaccgagtctggcaacccttccgccgacaccaagagaatcacctgtttcgcctctggcggcttccctaagcctcggttctcttggctggaaaacggcagagagctgcccggcatcaataccaccatttctcaggacccagagtccgagctgtacaccatctccagccagctcgactttaacaccaccagaaaccacaccatcaagtgcctgattaagtacggcgacgcccacgtgtccgaggactttacttgggagaaacctcctgaggaccctcctgactctggatctggcggcggaggttctggcggaggtggaagcggaggcggaggatctgctgagtctaagtatggccctccttgtcctccatgtcctgctccagaagctgctggcggaccctctgtgttcctgtttcctccaaagcctaaggaccagctcatgatctctcggacccctgaagtgacctgcgtggtggtggatgtgtctcaagaggaccctgaggtgcagttcaattggtacgtggacggcgtggaagtgcacaacgccaagaccaagcctagagaggaacagttcaactccacctatagagtggtgtccgtgctgaccgtgctgcaccaggattggctgaacggcaaagagtacaagtgcaaggtgtccaacaagggcctgccttccagcatcgaaaagaccatcagcaaggctaagggccagcctagggaaccccaggtttacaccctgcctccaagccaagaggaaatgaccaagaaccaggtgtccctgacctgcctggtcaagggcttctacccttccgacattgccgtggaatgggagtccaatggccagcctgagaacaactacaagaccacacctcctgtgctggactccgacggctccttctttctgtactctcgcctgaccgtggacaagtctaggtggcaagagggcaacgtgttctcctgctctgtgctgcacgaggctctgcacaaccactacacccagaagtccctgtctctgtctcttggaggtggtggcggttctgcccctacctccagctctaccaagaaaacccagctccagttggagcatctgctgctggacctccagatgatcctgaatggcatcaacaattacaagaaccccaagctgaccgccatgctgaccgctaagttctacatgcccaagaaggccaccgagctgaagcacttgcagtgcctggaaagggaactgaagcccctggaagaagtgctgaatctggcccagtccaagaacttccacctgaggcctagggacctgatctccaacatcaacgtgatcgtgctggaactgaaaggctccgagacaaccttcatgtgcgagtacgccgacgagacagccaccatcgtggaatttctgaaccggtggatcaccttctgccagagcatcatctccacactgacc

SEQ ID NO: 34 - protein, 616 aa, Artificial Sequence
  fusion protein (mGI102-M61)
MDAMLRGLCCVLLLCGAVFVSPSHAVDEQLSKSVKDKVLLPCRYNSPHEDESEDRIYWQKHDKVVLSVIAGKLKVWPEYKNRTLYDNTTYSLIILGLVLSDRGTYSCVVQKKERGTYEVKHLALVKLSIKADFSTPNITESGNPSADTKRITCFASGGFPKPRFSWLENGRELPGINTTISQDPESELYTISSQLDFNTTRNHTIKCLIKYGDAHVSEDFTWEKPPEDPPDSGSGGGGSGGGGSGGGGSAESKYGPPCPPCPAPEAAGGPSVFLFPPKPKDQLMISRTPEVTCVVVDVSQEDPEVQFNWYVDGVEVHNAKTKPREEQFNSTYRVVSVLTVLHQDWLNGKEYKCKVSNKGLPSSIEKTISKAKGQPREPQVYTLPPSQEEMTKNQVSLTCLVKGFYPSDIAVEWESNGQPENNYKTTPPVLDSDGSFFLYSRLTVDKSRWQEGNVFSCSVLHEALHNHYTQKSLSLSLGGGGGSAPTSSSTKKTQLQLEHLLLDLQMILNGINNYKNPKLTAMLTAKFYMPKKATELKHLQCLERELKPLEEVLNLAQSKNFHLRPRDLISNINVIVLELKGSETTFMCEYADETATIVEFLNRWITFCQSIISTLT

SEQ ID NO: 35 - protein, 153 aa, Artificial Sequence
  wild type hIL-2
MYRMQLLSCIALSLALVTNSAPTSSSTKKTQLQLEHLLLDLQMILNGINNYKNPKLTRMLTFKFYMPKKATELKHLQCLEEELKPLEEVLNLAQSKNFHLRPRDLISNINVIVLELKGSETTFMCEYADETATIVEFLNRWITFCQSIISTLT

SEQ ID NO: 36 - protein, 158 aa, Artificial Sequence
  IL-2 with signal sequence
MDAMLRGLCCVLLLCGAVFVSPSHAAPTSSSTKKTQLQLEHLLLDLQMILNGINNYKNPKLTRMLTFKFYMPKKATELKHLQCLEEELKPLEEVLNLAQSKNFHLRPRDLISNINVIVLELKGSETTFMCEYADETATIVEFLNRWITFCQSIISTLT

SEQ ID NO: 37 - DNA, 474 bp, Artificial Sequence
  nucleotide sequence coding IL-2 with signal sequence
atggatgctatgctgagaggcctgtgttgcgtgctgctgctgtgtggcgctgtgttcgtgtctccttctcacgctgcccctaccagctcctctaccaagaaaacccagctccagttggagcatctgctgctggacctccagatgattctgaacgggatcaacaactataagaaccccaagctgacccgcatgctgacctttaagttctacatgcccaagaaggccaccgagctgaagcacctccagtgcctggaagaagaactgaagcccctggaagaggtgctgaatctggcccagtccaagaacttccacctgaggccacgggacctgatcagcaacatcaacgtgatcgtgctggaactgaagggctccgagacaacctttatgtgcgagtacgccgacgagacagccaccatcgtggaatttctgaaccggtggatcaccttctgccagagcatcatctccacactgacc

SEQ ID NO: 38 - protein, 591 aa, Artificial Sequence
  mGI-101
VDEQLSKSVKDKVLLPCRYNSPHEDESEDRIYWQKHDKVVLSVIAGKLKVWPEYKNRTLYDNTTYSLIILGLVLSDRGTYSCVVQKKERGTYEVKHLALVKLSIKADFSTPNITESGNPSADTKRITCFASGGFPKPRFSWLENGRELPGINTTISQDPESELYTISSQLDFNTTRNHTIKCLIKYGDAHVSEDFTWEKPPEDPPDSGSGGGGSGGGGSGGGGSAESKYGPPCPPCPAPEAAGGPSVFLFPPKPKDQLMISRTPEVTCVVVDVSQEDPEVQFNWYVDGVEVHNAKTKPREEQFNSTYRVVSVLTVLHQDWLNGKEYKCKVSNKGLPSSIEKTISKAKGQPREPQVYTLPPSQEEMTKNQVSLTCLVKGFYPSDIAVEWESNGQPENNYKTTPPVLDSDGSFFLYSRLTVDKSRWQEGNVFSCSVLHEALHNHYTQKSLSLSLGGGGGSAPTSSSTKKTQLQLEHLLLDLQMILNGINNYKNPKLTAMLTAKFYMPKKATELKHLQCLEEELKPLEEVLNLAQSKNFHLRPRDLISNINVIVLELKGSETTFMCEYADETATIVEFLNRWITFCQSIISTLT

SEQ ID NO: 39 - protein, 120 aa, Artificial Sequence
  TIGIT ECD
MMTGTIETTGNISAEKGGSIILQCHLSSTTAQVTQVNWEQQDQLLAICNADLGWHISPSFKDRVAPGPGLGLTLQSLTVNDTGEYFCIYHTYPDGTYTGRIFLEVLESSVAEHGARFQIP